European Patent Specification EP 3 707 159 B1, published January 4, 2023. Title: NOVEL ENGINEERED T CELL RECEPTORS AND IMMUNE THERAPY USING THE SAME. Applicant: Immatics Biotechnologies GmbH. The sequence listing filed with the application follows.

SEQUENCE LISTING (66 sequences)

SEQ ID NO: 1 - protein, 9 aa, Homo sapiens
FLLDGSANV

SEQ ID NO: 2 - protein, 274 aa, Homo sapiens
MKSLRVLLVILWLQLSWVWSQQKEVEQNSGPLSVPEGAIASLNCTYSDRGSQSFFWYRQYSGKSPELIMFIYSNGDKEDGRFTAQLNKASQYVSLLIRDSQPSDSATYLCAAYSGAGSYQLTFGKGTKLSVIPNIQNPDPAVYQLRDSKSSDKSVCLFTDFDSQTNVSQSKDSDVYITDKTVLDMRSMDFKSNSAVAWSNKSDFACANAFNNSIIPEDTFFPSPESSCDVKLVEKSFETDTNLNFQNLSVIGFRILLLKVAGFNLLMTLRLWSS

SEQ ID NO: 3 - protein, 21 aa, Homo sapiens
MKSLRVLLVILWLQLSWVWSQ

SEQ ID NO: 4 - protein, 112 aa, Homo sapiens
QKEVEQNSGPLSVPEGAIASLNCTYSDRGSQSFFWYRQYSGKSPELIMFIYSNGDKEDGRFTAQLNKASQYVSLLIRDSQPSDSATYLCAAYSGAGSYQLTFGKGTKLSVIP

SEQ ID NO: 5 - protein, 6 aa, Homo sapiens
DRGSQS

SEQ ID NO: 6 - protein, 5 aa, Homo sapiens
YSNGD

SEQ ID NO: 7 - protein, 13 aa, Homo sapiens
CAAYSGAGSYQLT

SEQ ID NO: 8 - protein, 141 aa, Homo sapiens
NIQNPDPAVYQLRDSKSSDKSVCLFTDFDSQTNVSQSKDSDVYITDKTVLDMRSMDFKSNSAVAWSNKSDFACANAFNNSIIPEDTFFPSPESSCDVKLVEKSFETDTNLNFQNLSVIGFRILLLKVAGFNLLMTLRLWSS

SEQ ID NO: 9 - protein, 4 aa, Homo sapiens
NIQN

SEQ ID NO: 10 - protein, 308 aa, Homo sapiens
MGFRLLCCVAFCLLGAGPVDSGVTQTPKHLITATGQRVTLRCSPRSGDLSVYWYQQSLDQGLQFLIQYYNGEERAKGNILERFSAQQFPDLHSELNLSSLELGDSALYFCASSVESSYGYTFGSGTRLTVVEDLNKVFPPEVAVFEPSEAEISHTQKATLVCLATGFFPDHVELSWWVNGKEVHSGVSTDPQPLKEQPALNDSRYCLSSRLRVSATFWQNPRNHFRCQVQFYGLSENDEWTQDRAKPVTQIVSAEAWGRADCGFTSVSYQQGVLSATILYEILLGKATLYAVLVSALVLMAMVKRKDF

SEQ ID NO: 11 - protein, 19 aa, Homo sapiens
MGFRLLCCVAFCLLGAGPV

SEQ ID NO: 12 - protein, 112 aa, Homo sapiens
DSGVTQTPKHLITATGQRVTLRCSPRSGDLSVYWYQQSLDQGLQFLIQYYNGEERAKGNILERFSAQQFPDLHSELNLSSLELGDSALYFCASSVESSYGYTFGSGTRLTVV

SEQ ID NO: 13 - protein, 6 aa, Homo sapiens
RSGDLS

SEQ ID NO: 14 - protein, 5 aa, Homo sapiens
YNGEE

SEQ ID NO: 15 - protein, 12 aa, Homo sapiens
CASSVESSYGYT

SEQ ID NO: 16 - protein, 177 aa, Homo sapiens
EDLNKVFPPEVAVFEPSEAEISHTQKATLVCLATGFFPDHVELSWWVNGKEVHSGVSTDPQPLKEQPALNDSRYCLSSRLRVSATFWQNPRNHFRCQVQFYGLSENDEWTQDRAKPVTQIVSAEAWGRADCGFTSVSYQQGVLSATILYEILLGKATLYAVLVSALVLMAMVKRKDF

SEQ ID NO: 17 - protein, 5 aa, Homo sapiens
EDLNK

SEQ ID NO: 18 - protein, 5 aa, Homo sapiens
EDLKN

SEQ ID NO: 19 - protein, 374 aa, Homo sapiens
MQLLRCFSIFSVIASVLAQELTTICEQIPSPTLESTPYSLSTTTILANGKAMQGVFEYYKSVTFVSNCGSHPSTTSKGSPINTQYVFGGGGSDYKDDDDKGGGASQKEVEQNSGPLSVPEGAIASLNCTYSDRGSQSFFWYRQYSGKSPELIMSIYSNGDKEDGRFTAQLNKASQYVSLLIRDSQPSDSATYLCAAYSGAGSYQLTFGKGTKLSVIPNIQNGGGGSGGGGSGGGGSGGGGSGVTQTPKHLITATGQRVTLRCSPRSGDLSVYWYQQSLDQGLQFLIQYYNGEERAKGNILERFSAQQFPDLHSELNLSSLELGDSALYFCASSVESSYGYTFGSGTRLTVVEDLNKAAAGGSGGEQKLISEEDL

SEQ ID NO: 20 - protein, 87 aa, Homo sapiens
MQLLRCFSIFSVIASVLAQELTTICEQIPSPTLESTPYSLSTTTILANGKAMQGVFEYYKSVTFVSNCGSHPSTTSKGSPINTQYVF

SEQ ID NO: 21 - protein, 18 aa, Homo sapiens
GGGGSDYKDDDDKGGGAS

SEQ ID NO: 22 - protein, 251 aa, Homo sapiens
QKEVEQNSGPLSVPEGAIASLNCTYSDRGSQSFFWYRQYSGKSPELIMSIYSNGDKEDGRFTAQLNKASQYVSLLIRDSQPSDSATYLCAAYSGAGSYQLTFGKGTKLSVIPNIQNGGGGSGGGGSGGGGSGGGGSGVTQTPKHLITATGQRVTLRCSPRSGDLSVYWYQQSLDQGLQFLIQYYNGEERAKGNILERFSAQQFPDLHSELNLSSLELGDSALYFCASSVESSYGYTFGSGTRLTVVEDLNK

SEQ ID NO: 23 - protein, 18 aa, Homo sapiens
AAAGGSGGEQKLISEEDL

SEQ ID NO: 24 - protein, 251 aa, Homo sapiens
QKEVEQNSGPLSVPEGAIASLNCTYSDRGSQSFFWYRQYSGKSPELIMSIYSNGDKEDGRFTAQLNKASQYVSLLIRDSQPSDSATYLCAAYSGAGSYQLTFGKGTKLSVIPNIQNGGGGSGGGGSGGGGSGGGGSGVTQTPKHLITATGQRVTLRCSPRSGDLSVYWYKQSLDQGLQFLIQYYNGEERAKGNILERFSAQQFPDLHSELNLSSLELGDSALYFCASSVESSYGYTFGSGTRLTVVEDLNK

SEQ ID NO: 25 - protein, 251 aa, Homo sapiens
QKEVEQNSGPLSVPEGAIASLNCTYSDRGSQSFFWYRQYSGKSPELIMSIYSNGDKEDGRFTAQLNKASQYVSLLIRDSQPSDSATYLCAAYSGAGSYQLTFGKGTKLSVIPNIQNGGGGSGGGGSGGGGSGGGGSGVTQTPKHLITATGQRVTLRCSPRSGDLSVYWYQQSLDQGLQFLIQYYNGEERAKGNISERFSAQQFPDLHSELNLSSLELGDSALYFCASSVESSYGYTFGSGTRLTVVEDLNK

SEQ ID NO: 26 - protein, 6 aa, Homo sapiens
DRRSQS

SEQ ID NO: 27 - protein, 247 aa, Homo sapiens
QKEVEQNSGPLSVPEGAIASLNCTYSDRRSQSFFWYRQYSGKSPELIMSIYSNGDKEDGRFTAQLNKASQYVSLLIRDSQPSDSATYLCAAYSGAGSYQLTFGKGTKLSVIPGGGGSGGGGSGGGGSGGGGSGGGGSGVTQTPKHLITATGQRVTLRCSPRSGDLSVYWYKQSLDQGLQFLIQYYNGEERAKGNISERFSAQQFPDLHSELNLSSLELGDSALYFCASSVESSYGYTFGSGTRLTVV

SEQ ID NO: 28 - protein, 9 aa, Homo sapiens
ALLDGRVQL

SEQ ID NO: 29 - protein, 9 aa, Homo sapiens
RLLDGAFKL

SEQ ID NO: 30 - protein, 9 aa, Homo sapiens
ILLDGSASV

SEQ ID NO: 31 - protein, 9 aa, Homo sapiens
FLLDGSERL

SEQ ID NO: 32 - protein, 10 aa, Homo sapiens
FLFDGSANLV

SEQ ID NO: 33 - protein, 9 aa, Homo sapiens
FLFDGSANL

SEQ ID NO: 34 - protein, 9 aa, Homo sapiens
FLLDGSEGV

SEQ ID NO: 35 - protein, 9 aa, Homo sapiens
FLLDGSNSV

SEQ ID NO: 36 - protein, 9 aa, Homo sapiens
FLLDGSSRL

SEQ ID NO: 37 - protein, 6 aa, Homo sapiens
ARWHNN

SEQ ID NO: 38 - protein, 6 aa, Homo sapiens
AKDHLN

SEQ ID NO: 39 - protein, 6 aa, Homo sapiens
ARWHRN

SEQ ID NO: 40 - protein, 6 aa, Homo sapiens
AMDHPY

SEQ ID NO: 41 - protein, 6 aa, Homo sapiens
ATDHYN

SEQ ID NO: 42 - protein, 6 aa, Homo sapiens
ARYHTN

SEQ ID NO: 43 - protein, 6 aa, Homo sapiens
APYHLN

SEQ ID NO: 44 - protein, 6 aa, Homo sapiens
AKDHTN

SEQ ID NO: 45 - protein, 6 aa, Homo sapiens
ARYHRN

SEQ ID NO: 46 - protein, 6 aa, Homo sapiens
ARWHSN

SEQ ID NO: 47 - protein, 6 aa, Homo sapiens
ATDHYN

SEQ ID NO: 48 - protein, 6 aa, Homo sapiens
RWGDLN

SEQ ID NO: 49 - protein, 6 aa, Homo sapiens
ARDHLN

SEQ ID NO: 50 - protein, 514 aa, Homo sapiens
MKWVTFISLLFLFSSAYEVQLVESGGGLVQPGGSLRLSCAASGYSFTGYTMNWVRQAPGKGLEWVALINPYKGVSTYNQKFKDRFTISVDKSKNTAYLQMNSLRAEDTAVYYCARSGYYGDSDWYFDVWGQGTLVTVSSASTKGPSVFPLAPSSKSTSGGTAALGCLVKDYFPEPVTVSWNSGALTSGVHTFPAVLQSSGLYSLSSVVTVPSSSLGTQTYICNVNHKPSNTKVDKKVEPKSCDKTHTSPPSPAPPVAGQKEVEQNSGPLSVPEGAIASLNCTYSDRGSQSFFWYRQYSGKSPELIMSIYSNGDKEDGRFTAQLNKASQYVSLLIRDSQPSDSATYLCAAYSGAGSYQLTFGKGTKLSVIPNIQNGGGGSGGGGSGGGGSGGGGSGGGGSGVTQTPKHLITATGQRVTLRCSPRSGDLSVYWYKQSLDQGLQFLIQYYNGEERAKGNISERFSAQQFPDLHSELNLSSLELGDSALYFCASSVESSYGYTFGSGTRLTVVEDLKN

SEQ ID NO: 51 - protein, 258 aa, Homo sapiens
MKWVTFISLLFLFSSAYEVQLVESGGGLVQPGGSLRLSCAASGYSFTGYTMNWVRQAPGKGLEWVALINPYKGVSTYNQKFKDRFTISVDKSKNTAYLQMNSLRAEDTAVYYCARSGYYGDSDWYFDVWGQGTLVTVSSASTKGPSVFPLAPSSKSTSGGTAALGCLVKDYFPEPVTVSWNSGALTSGVHTFPAVLQSSGLYSLSSVVTVPSSSLGTQTYICNVNHKPSNTKVDKKVEPKSCDKTHTSPPSPAPPVAG

SEQ ID NO: 52 - protein, 232 aa, Homo sapiens
MKWVTFISLLFLFSSAYSDIQMTQSPSSLSASVGDRVTITCRASQDIRNYLNWYQQKPGKAPKLLIYYTSRLESGVPSRFSGSGSGTDYTLTISSLQPEDFATYYCQQGNTLPWTFGQGTKVEIKRTVAAPSVFIFPPSDEQLKSGTASVVCLLNNFYPREAKVQWKVDNALQSGNSQESVTEQDSKDSTYSLSSTLTLSKADYEKHKVYACEVTHQGLSSPVTKSFNRGEC

SEQ ID NO: 53 - protein, 274 aa, Homo sapiens
METLLGLLILWLQLQWVSSKQEVTQIPAALSVPEGENLVLNCSFTDSAIYNLQWFRQDPGKGLTSLLLIQSSQREQTSGRLNASLDKSSGRSTLYIAASQPGDSATYLCAVRPTSGGSYIPTFGRGTSLIVHPYIQNPDPAVYQLRDSKSSDKSVCLFTDFDSQTNVSQSKDSDVYITDKTVLDMRSMDFKSNSAVAWSNKSDFACANAFNNSIIPEDTFFPSPESSCDVKLVEKSFETDTNLNFQNLSVIGFRILLLKVAGFNLLMTLRLWSS

SEQ ID NO: 54 - protein, 20 aa, Homo sapiens
METLLGLLILWLQLQWVSSK

SEQ ID NO: 55 - protein, 113 aa, Homo sapiens
QEVTQIPAALSVPEGENLVLNCSFTDSAIYNLQWFRQDPGKGLTSLLLIQSSQREQTSGRLNASLDKSSGRSTLYIAASQPGDSATYLCAVRPTSGGSYIPTFGRGTSLIVHP

SEQ ID NO: 56 - protein, 141 aa, Homo sapiens
YIQNPDPAVYQLRDSKSSDKSVCLFTDFDSQTNVSQSKDSDVYITDKTVLDMRSMDFKSNSAVAWSNKSDFACANAFNNSIIPEDTFFPSPESSCDVKLVEKSFETDTNLNFQNLSVIGFRILLLKVAGFNLLMTLRLWSS

SEQ ID NO: 57 - protein, 311 aa, Homo sapiens
MSIGLLCCAALSLLWAGPVNAGVTQTPKFQVLKTGQSMTLQCAQDMNHEYMSWYRQDPGMGLRLIHYSVGAGITDQGEVPNGYNVSRSTTEDFPLRLLSAAPSQTSVYFCASSYVGNTGELFFGEGSRLTVLEDLKNVFPPEVAVFEPSEAEISHTQKATLVCLATGFYPDHVELSWWVNGKEVHSGVSTDPQPLKEQPALNDSRYCLSSRLRVSATFWQNPRNHFRCQVQFYGLSENDEWTQDRAKPVTQIVSAEAWGRADCGFTSESYQQGVLSATILYEILLGKATLYAVLVSALVLMAMVKRKDSRG

SEQ ID NO: 58 - protein, 21 aa, Homo sapiens
MSIGLLCCAALSLLWAGPVNA

SEQ ID NO: 59 - protein, 111 aa, Homo sapiens
GVTQTPKFQVLKTGQSMTLQCAQDMNHEYMSWYRQDPGMGLRLIHYSVGAGITDQGEVPNGYNVSRSTTEDFPLRLLSAAPSQTSVYFCASSYVGNTGELFFGEGSRLTVL

SEQ ID NO: 60 - protein, 179 aa, Homo sapiens
EDLKNVFPPEVAVFEPSEAEISHTQKATLVCLATGFYPDHVELSWWVNGKEVHSGVSTDPQPLKEQPALNDSRYCLSSRLRVSATFWQNPRNHFRCQVQFYGLSENDEWTQDRAKPVTQIVSAEAWGRADCGFTSESYQQGVLSATILYEILLGKATLYAVLVSALVLMAMVKRKDSRG

SEQ ID NO: 61 - protein, 9 aa, Homo sapiens
SLLMWITQV

SEQ ID NO: 62 - protein, 308 aa, Homo sapiens
MGFRLLCCVAFCLLGAGPVDSGVTQTPKHLITATGQRVTLRCSPAMDHPYVYWYQQSLDQGLQFLIQYYNGEERAKGNILERFSAQQFPDLHSELNLSSLELGDSALYFCASSVESSYGYTFGSGTRLTVVEDLNKVFPPEVAVFEPSEAEISHTQKATLVCLATGFFPDHVELSWWVNGKEVHSGVSTDPQPLKEQPALNDSRYCLSSRLRVSATFWQNPRNHFRCQVQFYGLSENDEWTQDRAKPVTQIVSAEAWGRADCGFTSVSYQQGVLSATILYEILLGKATLYAVLVSALVLMAMVKRKDF

SEQ ID NO: 63 - protein, 274 aa, Homo sapiens
MKSLRVLLVILWLQLSWVWSQQKEVEQNSGPLSVPEGAIASLNCTYSDRRSQSFFWYRQYSGKSPELIMFIYSNGDKEDGRFTAQLNKASQYVSLLIRDSQPSDSATYLCAAYSGAGSYQLTFGKGTKLSVIPNIQNPDPAVYQLRDSKSSDKSVCLFTDFDSQTNVSQSKDSDVYITDKTVLDMRSMDFKSNSAVAWSNKSDFACANAFNNSIIPEDTFFPSPESSCDVKLVEKSFETDTNLNFQNLSVIGFRILLLKVAGFNLLMTLRLWSS

SEQ ID NO: 64 - protein, 515 aa, Homo sapiens
MKWVTFISLLFLFSSAYSEVQLVESGGGLVQPGGSLRLSCAASGYSFTGYTMNWVRQAPGKGLEWVALINPYKGVSTYNQKFKDRFTISVDKSKNTAYLQMNSLRAEDTAVYYCARSGYYGDSDWYFDVWGQGTLVTVSSASTKGPSVFPLAPSSKSTSGGTAALGCLVKDYFPEPVTVSWNSGALTSGVHTFPAVLQSSGLYSLSSVVTVPSSSLGTQTYICNVNHKPSNTKVDKKVEPKSCDKTHTSPPSPAPPVAGQKEVEQNSGPLSVPEGAIASLNCTYSDRGSQSFFWYRQYSGKSPELIMSIYSNGDKEDGRFTAQLNKASQYVSLLIRDSQPSDSATYLCAAYSGAGSYQLTFGKGTKLSVIPNIQNGGGGSGGGGSGGGGSGGGGSGGGGSGVTQTPKHLITATGQRVTLRCSPAMDHPYVYWYKQSLDQGLQFLIQYYNGEERAKGNISERFSAQQFPDLHSELNLSSLELGDSALYFCASSVESSYGYTFGSGTRLTVVEDLKN

SEQ ID NO: 65 - protein, 515 aa, Homo sapiens
MKWVTFISLLFLFSSAYSEVQLVESGGGLVQPGGSLRLSCAASGYSFTGYTMNWVRQAPGKGLEWVALINPYKGVSTYNQKFKDRFTISVDKSKNTAYLQMNSLRAEDTAVYYCARSGYYGDSDWYFDVWGQGTLVTVSSASTKGPSVFPLAPSSKSTSGGTAALGCLVKDYFPEPVTVSWNSGALTSGVHTFPAVLQSSGLYSLSSVVTVPSSSLGTQTYICNVNHKPSNTKVDKKVEPKSCDKTHTSPPSPAPPVAGQKEVEQNSGPLSVPEGAIASLNCTYSDRRSQSFFWYRQYSGKSPELIMSIYSNGDKEDGRFTAQLNKASQYVSLLIRDSQPSDSATYLCAAYSGAGSYQLTFGKGTKLSVIPNIQNGGGGSGGGGSGGGGSGGGGSGGGGSGVTQTPKHLITATGQRVTLRCSPAMDHPYVYWYKQSLDQGLQFLIQYYNGEERAKGNISERFSAQQFPDLHSELNLSSLELGDSALYFCASSVESSYGYTFGSGTRLTVVEDLKN

SEQ ID NO: 66 - protein, 515 aa, Homo sapiens
MKWVTFISLLFLFSSAYSEVQLVESGGGLVQPGGSLRLSCAASGYSFTGYTMNWVRQAPGKGLEWVALINPYKGVSTYNQKFKDRFTISVDKSKNTAYLQMNSLRAEDTAVYYCARSGYYGDSDWYFDVWGQGTLVTVSSASTKGPSVFPLAPSSKSTSGGTAALGCLVKDYFPEPVTVSWNSGALTSGVHTFPAVLQSSGLYSLSSVVTVPSSSLGTQTYICNVNHKPSNTKVDKKVEPKSCDKTHTSPPSPAPPVAGGVTQTPKHLITATGQRVTLRCSPRSGDLSVYWYKQSLDQGLQFLIQYYNGEERAKGNISERFSAQQFPDLHSELNLSSLELGDSALYFCASSVESSYGYTFGSGTRLTVVEDLKNGGGGSGGGGSGGGGSGGGGSGGGGSQKEVEQNSGPLSVPEGAIASLNCTYSDRRSQSFFWYRQYSGKSPELIMSIYSNGDKEDGRFTAQLNKASQYVSLLIRDSQPSDSATYLCAAYSGAGSYQLTFGKGTKLSVIPNIQN